European Patent Application EP 4 656 244 A2, published December 3, 2025. Title: Gene therapy for ocular diseases. Applicant: The Trustees of The University of Pennsylvania. Application EP. The sequence listing filed with the application follows.

SEQUENCE LISTING (15 sequences)

SEQ ID NO: 1 - protein, 697 aa, Homo sapiens
MGERAGSPGTDQERKAGKHHYSYLSDFETPQSSGRSSLVSSSPASVRRKNPKRQTSDGQVHHQAPRKPSPKGLPNRKGVRVGFRSQSLNREPLRKDTDLVTKRILSARLLKINELQNEVSELQVKLAELLKENKSLKRLQYRQEKALNKFEDAENEISQLIFRHNNEITALKERLRKSQEKERATEKRVKDTESELFRTKFSLQKLKEISEARHLPERDDLAKKLVSAELKLDDTERRIKELSKNLELSTNSFQRQLLAERKRAYEAHDENKVLQKEVQRLYHKLKEKERELDIKNIYSNRLPKSSPNKEKELALRKNAACQSDFADLCTKGVQTMEDFKPEEYPLTPETIMCYENKWEEPGHLTLDLQSQKQDRHGEAGILNPIMEREEKFVTDEELHVVKQEVEKLEDEWEREELDKKQKEKASLLEREEKPEWETGRYQLGMYPIQNMDKLQGEEEERLKREMLLAKLNEIDRELQDSRNLKYPVLPLLPDFESKLHSPERSPKTYRFSESSERLFNGHHLQDISFSTPKGEGQNSGNVRSPASPNEFAFGSYVPSFAKTSERSNPFSQKSSFLDFQRNSMEKLSKDGVDLITRKEKKANLMEQLFGASGSSTISSKSSDPNSVASSKGDIDPLNFLPGNKGSRDQEHDEDEGFFLSEGRSFNPNRHRLKHADDKPAVKAADSVEDEIEEVALR

SEQ ID NO: 2 - DNA, 2094 bp, Homo sapiens
  source 1..2094: mol_type = genomic DNA
atgggggaaagagcaggaagtccaggtactgaccaagaaagaaaggcaggcaaacaccattattcttacttatctgattttgaaacgccacagtcttctggccgatcatcgctggtcagttcttcacctgcaagtgttaggagaaaaaatcctaaaagacaaacttcagatggccaagtacatcaccaagcccctcggaaaccaagccccaagggtctaccaaacagaaagggagtccgagtgggatttcgctcccagagcctcaatagagagccacttcggaaagatactgatcttgttacaaaacggattctgtctgcaagactgctaaaaatcaatgagttgcagaatgaagtatctgaactccaggtcaagttagctgagctgctaaaagaaaataaatctttgaaaaggcttcagtacagacaggagaaagccctgaataagtttgaagatgccgaaaatgaaatctcacaacttatatttcgtcataacaatgagattacagcactcaaagaacgcttaagaaaatctcaagagaaagaacgggcaactgagaaaagggtaaaagatacagaaagtgaactatttaggacaaaattttccttacagaaactgaaagagatctctgaagctagacacctacctgaacgagatgatttggcaaagaaactagtttcagcagagttaaagttagatgacaccgagagaagaattaaggagctatcgaaaaaccttgaactgagtactaacagtttccaacgacagttgcttgctgaaaggaaaagggcatatgaggctcatgatgaaaataaagttcttcaaaaggaggtacagcgactatatcacaaattaaaggaaaaggagagagaactggatataaaaaatatatattctaatcgtctgccaaagtcctctccaaataaagagaaagaacttgcattaagaaaaaatgctgcatgccagagtgattttgcagacctgtgtacaaaaggagtacaaaccatggaagacttcaagccagaagaatatcctttaactccagaaacaattatgtgttacgaaaacaaatgggaagaaccaggacatcttactttggacttgcaatctcaaaagcaagacaggcatggagaagcagggattctaaacccaattatggaaagagaagaaaaatttgttacagatgaagaactccatgtcgtaaaacaggaggttgaaaagctggaggatgaatgggaaagagaagaacttgataaaaagcaaaaagaaaaggcatctttactggaaagagaagaaaagccagagtgggaaactggaaggtaccaactaggaatgtatccaattcagaatatggataaattgcaaggagaggaagaagaaagactgaagagagaaatgctacttgctaaactgaatgaaattgacagagaactccaagattctcgaaatctaaaataccctgttttgccattgttacctgattttgaatcaaaactacactccccagagagaagccccaaaacatacaggttctctgaatcctcagagagattatttaatgggcatcatttgcaagacatcagtttctcaactccaaaaggagaaggtcagaattcaggaaatgttagaagtccagcctcccctaatgagttcgcatttggtagctacgtgccttcgtttgcaaaaacatcagagaggtcaaatccatttagtcaaaaaagtagttttttggatttccaaagaaacagtatggaaaaacttagtaaagatggtgtagatttaattacaagaaaagagaaaaaagctaatttgatggaacagttatttggtgccagtggtagcagcaccatttcctccaaaagcagtgacccaaattctgtggcttccagtaaaggagacattgaccctctaaattttctccctgggaataaaggcagcagagatcaagaacatgatgaagatgaaggctttttcctcagtgaaggaagaagttttaatccaaataggcaccgattaaaacatgcagacgataaaccagcagtaaaagcagctgattctgtagaagatgaaattgaagaagtagcactgagatga

SEQ ID NO: 3 - DNA, 2093 bp, synthetic construct
  misc_feature 1..2093: note = constructed sequence
  source 1..2093: mol_type = other DNA
atgggagaacgagcaggcagccctggtacggaccaggaacgcaaggcggggaaacaccactatagctatttgtcagactttgagacaccgcagagctcgggtcggtcatccttggtgtcgtcaagcccggctagcgtccggcgaaagaatccaaagcgccaaacgtcagatggccaggtgcatcatcaggctccccggaaaccctcgcccaaaggattgccgaacagaaagggggtccgggtagggtttagatcgcagagcctgaatcgcgagcctcttagaaaagatacagaccttgtgactaagaggattctgtcggcacgactgttgaagattaacgaacttcagaatgaggtgtcagaactccaagtaaaacttgcggaactgcttaaggagaacaaatcgctcaagcggcttcagtatcgccaagagaaagcgctcaacaagttcgaggacgcggaaaacgagatttcgcagttgatctttaggcataacaacgagatcaccgcccttaaagaacgcttgcgcaaaagccaggagaaagaacgcgccacggagaagagggtcaaggacaccgaatcggaactgtttagaactaagttttcgcttcaaaagcttaaagaaatctcggaagcgaggcatctccctgagcgagatgatttggctaagaaacttgtatcggcagagctcaaattggatgatacggagaggaggattaaggaacttagcaaaaaccttgaattgtcaacgaactcgtttcaacggcagctgttggccgaaagaaaacgggcttatgaagcgcacgatgaaaacaaggtgctgcagaaagaggtgcagaggttgtaccataagctgaaagagaaggaaagagagctggacatcaaaaacatctacagcaaccggctgcctaagtcatcgccaaacaaagagaaagagctggcattgagaaagaatgcagcctgccagtcggattttgcggatctgtgcacgaaaggagtacagaccatggaggactttaagcccgaagaatacccacttacacccgagacaatcatgtgttacgagaacaagtgggaggagccgggacaccttactcttgatctccagagccaaaaacaggatcgccacggcgaggccggtattctcaacccgatcatggagagagaggagaagttcgtcacagatgaggagctccacgtcgtgaaacaagaagtggagaagctcgaggacgaatgggaacgagaagagcttgataagaagcagaaggagaaagcatcgttgctggaacgcgaagagaaaccggagtgggagactgggaggtatcagcttgggatgtacccaattcagaatatggacaaactccagggggaggaagaagagaggctcaagagggaaatgctcctggccaagttgaatgagattgaccgggagttgcaagactcacgcaacctcaagtaccctgtactccccctgcttccggattttgaatcaaaacttcactcccccgaacggagccccaagacctatcgattctcggaatcgtcggagagactcttcaatggacaccatttgcaagacatctccttttcaacacccaaaggggaaggccagaattccggaaatgtgcggtcgccagcgtcgccaaatgagttcgcattcggttcgtacgtgccctcattcgcgaaaacctcggagagatccaaccccttcagccaaaagtcgtcattcttggatttccagagaaactccatggaaaagctctccaaggatggagtcgatctcatcactagaaaagagaagaaggccaatctcatggaacagttgttcggagcgtcgggttcgtccaccatctcctccaagtcatcagaccccaattcggtcgcatcctcaaagggagacatcgaccctttgaatttcctgccgggaaacaagggttcgcgagatcaggaacatgacgaggacgaggggtttttcttgtccgaagggaggtccttcaatccgaatcgccacagattgaaacacgcggatgacaagcctgcggtgaaggctgcggactcagtagaggacgagatcgaggaagtggccctgagatg

SEQ ID NO: 4 - DNA, 2094 bp, Homo sapiens
  source 1..2094: mol_type = genomic DNA
atgggggaaagagcaggaagtccaggtactgatcaagaaagaaaggcaggcaaacaccattattcttacttatctgattttgaaacgccacagtcttctggccgatcatcgctggtcagttcttcacctgcaagtgttaggagaaaaaatcctaaaagacaaacttcagatggccaagtacatcaccaagcccctcggaaaccaagccctaagggtctaccaaacagaaagggagtccgagtgggatttcgctcccagagcctcaatagagagccacttcggaaagatactgatcttgttacaaaacggattctgtctgcaagactgctaaaaatcaatgagttgcagaatgaagtatctgaactccaggtcaagttagctgagctgctaaaagaaaataaatctttgaaaaggcttcagtacagacaggagaaagccctgaataagtttgaagatgccgaaaatgaaatctcacaacttatatttcgtcataacaatgagattacagcactcaaagaacgcttaagaaaatctcaagagaaagaacgggcaactgagaaaagggtaaaagatacagaaagtgaactatttaggacaaaattttccttacagaaactgaaagagatctctgaagctagacacctacctgaacgagatgatttggcaaagaaactagtttcagcagagttaaagttagatgacaccgagagaagaattaaggagctatcgaaaaaccttgaactgagtactaacagtttccaacgacagttgcttgctgaaaggaaaagggcatatgaggctcatgatgaaaataaagttcttcaaaaggaggtacagcgactatatcacaaattaaaggaaaaggagagagaactggatataaaaaatatatattctaatcgtctgccaaagtcctctccaaataaagagaaagaacttgcattaagaaaaaatgctgcatgccagagtgattttgcagacctgtgtacaaaaggagtacaaaccatggaagacttcaagccagaagaatatcctttaactccagaaacaattatgtgttacgaaaacaaatgggaagaaccaggacatcttactttggacttgcaatctcaaaagcaagacaggcatggagaagcagggattctaaacccaattatggaaagagaagaaaaatttgttacagatgaagaactccatgtcgtaaaacaggaggttgaaaagctggaggatgaatgggaaagagaagaacttgataaaaagcaaaaagaaaaggcatctttactggaaagagaagaaaagccagagtgggaaactggaaggtaccaactaggaatgtatccaattcagaatatggataaattgcaaggagaggaagaagaaagactgaagagagaaatgctacttgctaaactgaatgaaattgacagagaactccaagattctcgaaatctaaaataccctgttttgccattgttacctgattttgaatcaaaactacactccccagagagaagccccaaaacatacaggttctctgaatcctcagagagattatttaatgggcatcatttgcaagacatcagtttctcaactccaaaaggagaaggtcagaattcaggaaatgttagaagtccagcctcccctaatgagttcgcatttggtagctacgtgccttcgtttgcaaaaacatcagagaggtcaaatccatttagtcaaaaaagtagttttttggatttccaaagaaacagtatggaaaaacttagtaaagatggtgtagatttaattacaagaaaagagaaaaaagctaatttgatggaacagttatttggtgccagtggtagcagcaccatttcctccaaaagcagtgacccaaattctgtggcttccagtaaaggagacattgaccctctaaattttctccctgggaataaaggcagcagagatcaagaacatgatgaagatgaaggctttttcctcagtgaaggaagaagttttaatccaaataggcaccgattaaaacatgcagacgataaaccagcagtaaaagcagctgattctgtagaagatgaaattgaagaagtagcactgagatga

SEQ ID NO: 5 - DNA, 2094 bp, Homo sapiens; identical to SEQ ID NO: 4
  source 1..2094: mol_type = genomic DNA

SEQ ID NO: 6 - DNA, 2094 bp, Homo sapiens; identical to SEQ ID NO: 4
  source 1..2094: mol_type = genomic DNA

SEQ ID NO: 7 - DNA, 2094 bp, Homo sapiens; identical to SEQ ID NO: 4
  source 1..2094: mol_type = genomic DNA

SEQ ID NO: 8 - DNA, 12231 bp, synthetic construct
  misc_feature 1..12231: note = constructed sequence
  source 1..12231: mol_type = other DNA
ctgcgcgctcgctcgctcactgaggccgcccgggcaaagcccgggcgtcgggcgacctttggtcgcccggcctcagtgagcgagcgagcgcgcagagagggagtggccaactccatcactaggggttccttgtagttaatgattaacccgccatgctacttatctacgtagcaagctagctagttattaatagtaatcaattacggggtcattagttcatagcccatatatggagttccgcgttacataacttacggtaaatggcccgcctggctgaccgcccaacgacccccgcccattgacgtcaataatgacgtatgttcccatagtaacgccaatagggactttccattgacgtcaatgggtggagtatttacggtaaactgcccacttggcagtacatcaagtgtatcatatgccaagtacgccccctattgacgtcaatgacggtaaatggcccgcctggcattatgcccagtacatgaccttatgggactttcctacttggcagtacatctacgtattagtcatcgctattaacatggtcgaggtgagccccacgttctgcttcactctccccatctcccccccctccccacccccaattttgtatttatttattttttaattattttgtgcagcgatgggggcggggggggggggggggcgcgcgccaggcggggcggggcggggcgaggggcggggcggggcgaggcggagaggtgcggcggcagccaatcagagcggcgcgctccgaaagtttccttttatggcgaggcggcggcggcggcggccctataaaaagcgaagcgcgcggcgggcggggagtcgctgcgacgctgccttcgccccgtgccccgctccgccgccgcctcgcgccgcccgccccggctctgactgaccgcgttactcccacaggtgagcgggcgggacggcccttctcctccgggctgtaattagcgcttggtttaatgacggcttgtttcttttctgtggctgcgtgaaagccttgaggggctccgggagggccctttgtgcggggggagcggctcggggggtgcgtgcgtgtgtgtgtgcgtggggagcgccgcgtgcggctccgcgctgcccggcggctgtgagcgctgcgggcgcggcgcggggctttgtgcgctccgcagtgtgcgcgaggggagcgcggccgggggcggtgccccgcggtgcggggggggctgcgaggggaacaaaggctgcgtgcggggtgtgtgcgtgggggggtgagcagggggtgtgggcgcgtcggtcgggctgcaaccccccctgcacccccctccccgagttgctgagcacggcccggcttcgggtgcggggctccgtacggggcgtggcgcggggctcgccgtgccgggcggggggtggcggcaggtgggggtgccgggcggggcggggccgcctcgggccggggagggctcgggggaggggcgcggcggcccccggagcgccggcggctgtcgaggcgcggcgagccgcagccattgccttttatggtaatcgtgcgagagggcgcagggacttcctttgtcccaaatctgtgcggagccgaaatctgggaggcgccgccgcaccccctctagcgggcgcggggcgaagcggtgcggcgccggcaggaaggaaatgggcggggagggccttcgtgcgtcgccgcgccgccgtccccttctccctctccagcctcggggctgtccgcggggggacggctgccttcgggggggacggggcagggcggggttcggcttctggcgtgtgaccggcggctctagacaattgtactaaccttcttctctttcctctcctgacaggttggtgtacactagcggccgaatagagaccatttttcaaaacaatgggagaacgagcaggcagccctggtacggaccaggaacgcaaggcggggaaacaccactatagctatttgtcagactttgagacaccgcagagctcgggtcggtcatccttggtgtcgtcaagcccggctagcgtccggcgaaagaatccaaagcgccaaacgtcagatggccaggtgcatcatcaggctccccggaaaccctcgcccaaaggattgccgaacagaaagggggtccgggtagggtttagatcgcagagcctgaatcgcgagcctcttagaaaagatacagaccttgtgactaagaggattctgtcggcacgactgttgaagattaacgaacttcagaatgaggtgtcagaactccaagtaaaacttgcggaactgcttaaggagaacaaatcgctcaagcggcttcagtatcgccaagagaaagcgctcaacaagttcgaggacgcggaaaacgagatttcgcagttgatctttaggcataacaacgagatcaccgcccttaaagaacgcttgcgcaaaagccaggagaaagaacgcgccacggagaagagggtcaaggacaccgaatcggaactgtttagaactaagttttcgcttcaaaagcttaaagaaatctcggaagcgaggcatctccctgagcgagatgatttggctaagaaacttgtatcggcagagctcaaattggatgatacggagaggaggattaaggaacttagcaaaaaccttgaattgtcaacgaactcgtttcaacggcagctgttggccgaaagaaaacgggcttatgaagcgcacgatgaaaacaaggtgctgcagaaagaggtgcagaggttgtaccataagctgaaagagaaggaaagagagctggacatcaaaaacatctacagcaaccggctgcctaagtcatcgccaaacaaagagaaagagctggcattgagaaagaatgcagcctgccagtcggattttgcggatctgtgcacgaaaggagtacagaccatggaggactttaagcccgaagaatacccacttacacccgagacaatcatgtgttacgagaacaagtgggaggagccgggacaccttactcttgatctccagagccaaaaacaggatcgccacggcgaggccggtattctcaacccgatcatggagagagaggagaagttcgtcacagatgaggagctccacgtcgtgaaacaagaagtggagaagctcgaggacgaatgggaacgagaagagcttgataagaagcagaaggagaaagcatcgttgctggaacgcgaagagaaaccggagtgggagactgggaggtatcagcttgggatgtacccaattcagaatatggacaaactccagggggaggaagaagagaggctcaagagggaaatgctcctggccaagttgaatgagattgaccgggagttgcaagactcacgcaacctcaagtaccctgtactccccctgcttccggattttgaatcaaaacttcactcccccgaacggagccccaagacctatcgattctcggaatcgtcggagagactcttcaatggacaccatttgcaagacatctccttttcaacacccaaaggggaaggccagaattccggaaatgtgcggtcgccagcgtcgccaaatgagttcgcattcggttcgtacgtgccctcattcgcgaaaacctcggagagatccaaccccttcagccaaaagtcgtcattcttggatttccagagaaactccatggaaaagctctccaaggatggagtcgatctcatcactagaaaagagaagaaggccaatctcatggaacagttgttcggagcgtcgggttcgtccaccatctcctccaagtcatcagaccccaattcggtcgcatcctcaaagggagacatcgaccctttgaatttcctgccgggaaacaagggttcgcgagatcaggaacatgacgaggacgaggggtttttcttgtccgaagggaggtccttcaatccgaatcgccacagattgaaacacgcggatgacaagcctgcggtgaaggctgcggactcagtagaggacgagatcgaggaagtggccctgagatgatcaggatctgcctcgactgtgccttctagttgccagccatctgttgtttgcccctcccccgtgccttccttgaccctggaaggtgccactcccactgtcctttcctaataaaatgaggaaattgcatcgcattgtctgagtaggtgtcattctattctggggggtggggtggggcaggacagcaagggggaggattgggaagacaatagcaggcatgctggggactcgagttctacgtagataagtagcatggcgggttaatcattaactacaaggaacccctagtgatggagttggccactccctctctgcgcgctcgctcgctcactgaggccgggcgaccaaaggtcgcccgacgcccgggctttgcccgggcggcctcagtgagcgagcgagcgcgcagccttaattaacctaaggaaaatgaagtgaagttcctatactttctagagaataggaacttctatagtgagtcgaataagggcgacacaaaatttattctaaatgcataataaatactgataacatcttatagtttgtattatattttgtattatcgttgacatgtataattttgatatcaaaaactgattttccctttattattttcgagatttattttcttaattctctttaacaaactagaaatattgtatatacaaaaaatcataaataatagatgaatagtttaattataggtgttcatcaatcgaaaaagcaacgtatcttatttaaagtgcgttgcttttttctcatttataaggttaaataattctcatatatcaagcaaagtgacaggcgcccttaaatattctgacaaatgctctttccctaaactccccccataaaaaaacccgccgaagcgggtttttacgttatttgcggattaacgattactcgttatcagaaccgcccagggggcccgagcttaacctttttatttgggggagagggaagtcatgaaaaaactaacctttgaaattcgatctccagcacatcagcaaaacgctattcacgcagtacagcaaatccttccagacccaaccaaaccaatcgtagtaaccattcaggaacgcaaccgcagcttagaccaaaacaggaagctatgggcctgcttaggtgacgtctctcgtcaggttgaatggcatggtcgctggctggatgcagaaagctggaagtgtgtgtttaccgcagcattaaagcagcaggatgttgttcctaaccttgccgggaatggctttgtggtaataggccagtcaaccagcaggatgcgtgtaggcgaatttgcggagctattagagcttatacaggcattcggtacagagcgtggcgttaagtggtcagacgaagcgagactggctctggagtggaaagcgagatggggagacagggctgcatgataaatgtcgttagtttctccggtggcaggacgtcagcatatttgctctggctaatggagcaaaagcgacgggcaggtaaagacgtgcattacgttttcatggatacaggttgtgaacatccaatgacatatcggtttgtcagggaagttgtgaagttctgggatataccgctcaccgtattgcaggttgatatcaacccggagcttggacagccaaatggttatacggtatgggaaccaaaggatattcagacgcgaatgcctgttctgaagccatttatcgatatggtaaagaaatatggcactccatacgtcggcggcgcgttctgcactgacagattaaaactcgttcccttcaccaaatactgtgatgaccatttcgggcgagggaattacaccacgtggattggcatcagagctgatgaaccgaagcggctaaagccaaagcctggaatcagatatcttgctgaactgtcagactttgagaaggaagatatcctcgcatggtggaagcaacaaccattcgatttgcaaataccggaacatctcggtaactgcatattctgcattaaaaaatcaacgcaaaaaatcggacttgcctgcaaagatgaggagggattgcagcgtgtttttaatgaggtcatcacgggatcccatgtgcgtgacggacatcgggaaacgccaaaggagattatgtaccgaggaagaatgtcgctggacggtatcgcgaaaatgtattcagaaaatgattatcaagccctgtatcaggacatggtacgagctaaaagattcgataccggctcttgttctgagtcatgcgaaatatttggagggcagcttgatttcgacttcgggagggaagctgcatgatgcgatgttatcggtgcggtgaatgcaaagaagataaccgcttccgaccaaatcaaccttactggaatcgatggtgtctccggtgtgaaagaacaccaacaggggtgttaccactaccgcaggaaaaggaggacgtgtggcgagacagcgacgaagtatcaccgacataatctgcgaaaactgcaaataccttccaacgaaacgcaccagaaataaacccaagccaatcccaaaagaatctgacgtaaaaaccttcaactacacggctcacctgtgggatatccggtggctaagacgtcgtgcgaggaaaacaaggtgattgaccaaaatcgaagttacgaacaagaaagcgtcgagcgagctttaacgtgcgctaactgcggtcagaagctgcatgtgctggaagttcacgtgtgtgagcactgctgcgcagaactgatgagcgatccgaatagctcgatgcacgaggaagaagatgatggctaaaccagcgcgaagacgatgtaaaaacgatgaatgccgggaatggtttcaccctgcattcgctaatcagtggtggtgctctccagagtgtggaaccaagatagcactcgaacgacgaagtaaagaacgcgaaaaagcggaaaaagcagcagagaagaaacgacgacgagaggagcagaaacagaaagataaacttaagattcgaaaactcgccttaaagccccgcagttactggattaaacaagcccaacaagccgtaaacgccttcatcagagaaagagaccgcgacttaccatgtatctcgtgcggaacgctcacgtctgctcagtgggatgccggacattaccggacaactgctgcggcacctcaactccgatttaatgaacgcaatattcacaagcaatgcgtggtgtgcaaccagcacaaaagcggaaatctcgttccgtatcgcgtcgaactgattagccgcatcgggcaggaagcagtagacgaaatcgaatcaaaccataaccgccatcgctggactatcgaagagtgcaaggcgatcaaggcagagtaccaacagaaactcaaagacctgcgaaatagcagaagtgaggccgcatgacgttctcagtaaaaaccattccagacatgctcgttgaagcatacggaaatcagacagaagtagcacgcagactgaaatgtagtcgcggtacggtcagaaaatacgttgatgataaagacgggaaaatgcacgccatcgtcaacgacgttctcatggttcatcgcggatggagtgaaagagatgcgctattacgaaaaaattgatggcagcaaataccgaaatatttgggtagttggcgatctgcacggatgctacacgaacctgatgaacaaactggatacgattggattcgacaacaaaaaagacctgcttatctcggtgggcgatttggttgatcgtggtgcagagaacgttgaatgcctggaattaatcacattcccctggttcagagctgtacgtggaaaccatgagcaaatgatgattgatggcttatcagagcgtggaaacgttaatcactggctgcttaatggcggtggctggttctttaatctcgattacgacaaagaaattctggctaaagctcttgcccataaagcagatgaacttccgttaatcatcgaactggtgagcaaagataaaaaatatgttatctgccacgccgattatccctttgacgaatacgagtttggaaagccagttgatcatcagcaggtaatctggaaccgcgaacgaatcagcaactcacaaaacgggatcgtgaaagaaatcaaaggcgcggacacgttcatctttggtcatacgccagcagtgaaaccactcaagtttgccaaccaaatgtatatcgataccggcgcagtgttctgcggaaacctaacattgattcaggtacagggagaaggcgcatgagactcgaaagcgtagctaaatttcattcgccaaaaagcccgatgatgagcgactcaccacgggccacggcttctgactctctttccggtactgatgtgatggctgctatggggatggcgcaatcacaagccggattcggtatggctgcattctgcggtaagcacgaactcagccagaacgacaaacaaaaggctatcaactatctgatgcaatttgcacacaaggtatcggggaaataccgtggtgtggcaaagcttgaaggaaatactaaggcaaaggtactgcaagtgctcgcaacattcgcttatgcggattattgccgtagtgccgcgacgccgggggcaagatgcagagattgccatggtacaggccgtgcggttgatattgccaaaacagagctgtgggggagagttgtcgagaaagagtgcggaagatgcaaaggcgtcggctattcaaggatgccagcaagcgcagcatatcgcgctgtgacgatgctaatcccaaaccttacccaacccacctggtcacgcactgttaagccgctgtatgacgctctggtggtgcaatgccacaaagaagagtcaatcgcagacaacattttgaatgcggtcacacgttagcagcatgattgccacggatggcaacatattaacggcatgatattgacttattgaataaaattgggtaaatttgactcaacgatgggttaattcgctcgttgtggtagtgagatgaaaagaggcggcgcttactaccgattccgcctagttggtcacttcgacgtatcgtctggaactccaaccatcgcaggcagagaggtctgcaaaatgcaatcccgaaacagttcgcaggtaatagttagagcctgcataacggtttcgggattttttatatctgcacaacaggtaagagcattgagtcgataatcgtgaagagtcggcgagcctggttagccagtgctctttccgttgtgctgaattaagcgaataccggaagcagaaccggatcaccaaatgcgtacaggcgtcatcgccgcccagcaacagcacaacccaaactgagccgtagccactgtctgtcctgaattcattagtaatagttacgctgcggccttttacacatgaccttcgtgaaagcgggtggcaggaggtcgcgctaacaacctcctgccgttttgcccgtgcatatcggtcacgaacaaatctgattactaaacacagtagcctggatttgttctatcagtaatcgaccttattcctaattaaatagagcaaatccccttattgggggtaagacatgaagatgccagaaaaacatgacctgttggccgccattctcgcggcaaaggaacaaggcatcggggcaatccttgcgtttgcaatggcgtaccttcgcggcagatataatggcggtgcgtttacaaaaacagtaatcgacgcaacgatgtgcgccattatcgcctggttcattcgtgaccttctcgacttcgccggactaagtagcaatctcgcttatataacgagcgtgtttatcggctacatcggtactgactcgattggttcgcttatcaaacgcttcgctgctaaaaaagccggagtagaagatggtagaaatcaataatcaacgtaaggcgttcctcgatatgctggcgtggtcggagggaactgataacggacgtcagaaaaccagaaatcatggttatgacgtcattgtaggcggagagctatttactgattactccgatcaccctcgcaaacttgtcacgctaaacccaaaactcaaatcaacaggcgcttaagactggccgtcgttttacaacacagaaagagtttgtagaaacgcaaaaaggccatccgtcaggggccttctgcttagtttgatgcctggcagttccctactctcgccttccgcttcctcgctcactgactcgctgcgctcggtcgttcggctgcggcgagcggtatcagctcactcaaaggcggtaatacggttatccacagaatcaggggataacgcaggaaagaacatgtgagcaaaaggccagcaaaaggccaggaaccgtaaaaaggccgcgttgctggcgtttttccataggctccgcccccctgacgagcatcacaaaaatcgacgctcaagtcagaggtggcgaaacccgacaggactataaagataccaggcgtttccccctggaagctccctcgtgcgctctcctgttccgaccctgccgcttaccggatacctgtccgcctttctcccttcgggaagcgtggcgctttctcatagctcacgctgtaggtatctcagttcggtgtaggtcgttcgctccaagctgggctgtgtgcacgaaccccccgttcagcccgaccgctgcgccttatccggtaactatcgtcttgagtccaacccggtaagacacgacttatcgccactggcagcagccactggtaacaggattagcagagcgaggtatgtaggcggtgctacagagttcttgaagtggtgggctaactacggctacactagaagaacagtatttggtatctgcgctctgctgaagccagttaccttcggaaaaagagttggtagctcttgatccggcaaacaaaccaccgctggtagcggtggtttttttgtttgcaagcagcagattacgcgcagaaaaaaaggatctcaagaagatcctttgatcttttctacggggtctgacgctcagtggaacgacgcgcgcgtaactcacgttaagggattttggtcatgagcttgcgccgtcccgtcaagtcagcgtaatgctctgcttttagaaaaactcatcgagcatcaaatgaaactgcaatttattcatatcaggattatcaataccatatttttgaaaaagccgtttctgtaatgaaggagaaaactcaccgaggcagttccataggatggcaagatcctggtatcggtctgcgattccgactcgtccaacatcaatacaacctattaatttcccctcgtcaaaaataaggttatcaagtgagaaatcaccatgagtgacgactgaatccggtgagaatggcaaaagtttatgcatttctttccagacttgttcaacaggccagccattacgctcgtcatcaaaatcactcgcatcaaccaaaccgttattcattcgtgattgcgcctgagcgaggcgaaatacgcgatcgctgttaaaaggacaattacaaacaggaatcgagtgcaaccggcgcaggaacactgccagcgcatcaacaatattttcacctgaatcaggatattcttctaatacctggaacgctgtttttccggggatcgcagtggtgagtaaccatgcatcatcaggagtacggataaaatgcttgatggtcggaagtggcataaattccgtcagccagtttagtctgaccatctcatctgtaacatcattggcaacgctacctttgccatgtttcagaaacaactctggcgcatcgggcttcccatacaagcgatagattgtcgcacctgattgcccgacattatcgcgagcccatttatacccatataaatcagcatccatgttggaatttaatcgcggcctcgacgtttcccgttgaatatggctcatattcttcctttttcaatattattgaagcatttatcagggttattgtctcatgagcggatacatatttgaatgtatttagaaaaataaacaaataggggtcagtgttacaaccaattaaccaattctgaacattatcgcgagcccatttatacctgaatatggctcataacaccccttgtttgcctggcggcagtagcgcggtggtcccacctgaccccatgccgaactcagaagtgaaacgccgtagcgccgatggtagtgtggggactccccatgcgagagtagggaactgccaggcatcaaataaaacgaaaggctcagtcgaaagactgggcctttcgcccgggctaattagggggtgtcgcccttattcgactctatagtgaagttcctattctctagaaagtataggaacttctgaagtggggtcgacttaattaagg

SEQ ID NO: 9 - DNA, 12220 bp, synthetic construct
  misc_feature 1..12220: note = constructed sequence
  source 1..12220: mol_type = other DNA
ctgcgcgctcgctcgctcactgaggccgcccgggcaaagcccgggcgtcgggcgacctttggtcgcccggcctcagtgagcgagcgagcgcgcagagagggagtggccaactccatcactaggggttccttgtagttaatgattaacccgccatgctacttatctacgtagcaagctagctagttattaatagtaatcaattacggggtcattagttcatagcccatatatggagttccgcgttacataacttacggtaaatggcccgcctggctgaccgcccaacgacccccgcccattgacgtcaataatgacgtatgttcccatagtaacgccaatagggactttccattgacgtcaatgggtggagtatttacggtaaactgcccacttggcagtacatcaagtgtatcatatgccaagtacgccccctattgacgtcaatgacggtaaatggcccgcctggcattatgcccagtacatgaccttatgggactttcctacttggcagtacatctacgtattagtcatcgctattaacatggtcgaggtgagccccacgttctgcttcactctccccatctcccccccctccccacccccaattttgtatttatttattttttaattattttgtgcagcgatgggggcggggggggggggggggcgcgcgccaggcggggcggggcggggcgaggggcggggcggggcgaggcggagaggtgcggcggcagccaatcagagcggcgcgctccgaaagtttccttttatggcgaggcggcggcggcggcggccctataaaaagcgaagcgcgcggcgggcggggagtcgctgcgacgctgccttcgccccgtgccccgctccgccgccgcctcgcgccgcccgccccggctctgactgaccgcgttactcccacaggtgagcgggcgggacggcccttctcctccgggctgtaattagcgcttggtttaatgacggcttgtttcttttctgtggctgcgtgaaagccttgaggggctccgggagggccctttgtgcggggggagcggctcggggggtgcgtgcgtgtgtgtgtgcgtggggagcgccgcgtgcggctccgcgctgcccggcggctgtgagcgctgcgggcgcggcgcggggctttgtgcgctccgcagtgtgcgcgaggggagcgcggccgggggcggtgccccgcggtgcggggggggctgcgaggggaacaaaggctgcgtgcggggtgtgtgcgtgggggggtgagcagggggtgtgggcgcgtcggtcgggctgcaaccccccctgcacccccctccccgagttgctgagcacggcccggcttcgggtgcggggctccgtacggggcgtggcgcggggctcgccgtgccgggcggggggtggcggcaggtgggggtgccgggcggggcggggccgcctcgggccggggagggctcgggggaggggcgcggcggcccccggagcgccggcggctgtcgaggcgcggcgagccgcagccattgccttttatggtaatcgtgcgagagggcgcagggacttcctttgtcccaaatctgtgcggagccgaaatctgggaggcgccgccgcaccccctctagcgggcgcggggcgaagcggtgcggcgccggcaggaaggaaatgggcggggagggccttcgtgcgtcgccgcgccgccgtccccttctccctctccagcctcggggctgtccgcggggggacggctgccttcgggggggacggggcagggcggggttcggcttctggcgtgtgaccggcggctctagacaattgtactaaccttcttctctttcctctcctgacaggttggtgtacactagcggccgccaccatgggggaaagagcaggaagtccaggtactgaccaagaaagaaaggcaggcaaacaccattattcttacttatctgattttgaaacgccacagtcttctggccgatcatcgctggtcagttcttcacctgcaagtgttaggagaaaaaatcctaaaagacaaacttcagatggccaagtacatcaccaagcccctcggaaaccaagccccaagggtctaccaaacagaaagggagtccgagtgggatttcgctcccagagcctcaatagagagccacttcggaaagatactgatcttgttacaaaacggattctgtctgcaagactgctaaaaatcaatgagttgcagaatgaagtatctgaactccaggtcaagttagctgagctgctaaaagaaaataaatctttgaaaaggcttcagtacagacaggagaaagccctgaataagtttgaagatgccgaaaatgaaatctcacaacttatatttcgtcataacaatgagattacagcactcaaagaacgcttaagaaaatctcaagagaaagaacgggcaactgagaaaagggtaaaagatacagaaagtgaactatttaggacaaaattttccttacagaaactgaaagagatctctgaagctagacacctacctgaacgagatgatttggcaaagaaactagtttcagcagagttaaagttagatgacaccgagagaagaattaaggagctatcgaaaaaccttgaactgagtactaacagtttccaacgacagttgcttgctgaaaggaaaagggcatatgaggctcatgatgaaaataaagttcttcaaaaggaggtacagcgactatatcacaaattaaaggaaaaggagagagaactggatataaaaaatatatattctaatcgtctgccaaagtcctctccaaataaagagaaagaacttgcattaagaaaaaatgctgcatgccagagtgattttgcagacctgtgtacaaaaggagtacaaaccatggaagacttcaagccagaagaatatcctttaactccagaaacaattatgtgttacgaaaacaaatgggaagaaccaggacatcttactttggacttgcaatctcaaaagcaagacaggcatggagaagcagggattctaaacccaattatggaaagagaagaaaaatttgttacagatgaagaactccatgtcgtaaaacaggaggttgaaaagctggaggatgaatgggaaagagaagaacttgataaaaagcaaaaagaaaaggcatctttactggaaagagaagaaaagccagagtgggaaactggaaggtaccaactaggaatgtatccaattcagaatatggataaattgcaaggagaggaagaagaaagactgaagagagaaatgctacttgctaaactgaatgaaattgacagagaactccaagattctcgaaatctaaaataccctgttttgccattgttacctgattttgaatcaaaactacactccccagagagaagccccaaaacatacaggttctctgaatcctcagagagattatttaatgggcatcatttgcaagacatcagtttctcaactccaaaaggagaaggtcagaattcaggaaatgttagaagtccagcctcccctaatgagttcgcatttggtagctacgtgccttcgtttgcaaaaacatcagagaggtcaaatccatttagtcaaaaaagtagttttttggatttccaaagaaacagtatggaaaaacttagtaaagatggtgtagatttaattacaagaaaagagaaaaaagctaatttgatggaacagttatttggtgccagtggtagcagcaccatttcctccaaaagcagtgacccaaattctgtggcttccagtaaaggagacattgaccctctaaattttctccctgggaataaaggcagcagagatcaagaacatgatgaagatgaaggctttttcctcagtgaaggaagaagttttaatccaaataggcaccgattaaaacatgcagacgataaaccagcagtaaaagcagctgattctgtagaagatgaaattgaagaagtagcactgagatgatcataactgcagatctgcctcgactgtgccttctagttgccagccatctgttgtttgcccctcccccgtgccttccttgaccctggaaggtgccactcccactgtcctttcctaataaaatgaggaaattgcatcgcattgtctgagtaggtgtcattctattctggggggtggggtggggcaggacagcaagggggaggattgggaagacaatagcaggcatgctggggactcgagttctacgtagataagtagcatggcgggttaatcattaactacaaggaacccctagtgatggagttggccactccctctctgcgcgctcgctcgctcactgaggccgggcgaccaaaggtcgcccgacgcccgggctttgcccgggcggcctcagtgagcgagcgagcgcgcagccttaattaacctaaggaaaatgaagtgaagttcctatactttctagagaataggaacttctatagtgagtcgaataagggcgacacaaaatttattctaaatgcataataaatactgataacatcttatagtttgtattatattttgtattatcgttgacatgtataattttgatatcaaaaactgattttccctttattattttcgagatttattttcttaattctctttaacaaactagaaatattgtatatacaaaaaatcataaataatagatgaatagtttaattataggtgttcatcaatcgaaaaagcaacgtatcttatttaaagtgcgttgcttttttctcatttataaggttaaataattctcatatatcaagcaaagtgacaggcgcccttaaatattctgacaaatgctctttccctaaactccccccataaaaaaacccgccgaagcgggtttttacgttatttgcggattaacgattactcgttatcagaaccgcccagggggcccgagcttaacctttttatttgggggagagggaagtcatgaaaaaactaacctttgaaattcgatctccagcacatcagcaaaacgctattcacgcagtacagcaaatccttccagacccaaccaaaccaatcgtagtaaccattcaggaacgcaaccgcagcttagaccaaaacaggaagctatgggcctgcttaggtgacgtctctcgtcaggttgaatggcatggtcgctggctggatgcagaaagctggaagtgtgtgtttaccgcagcattaaagcagcaggatgttgttcctaaccttgccgggaatggctttgtggtaataggccagtcaaccagcaggatgcgtgtaggcgaatttgcggagctattagagcttatacaggcattcggtacagagcgtggcgttaagtggtcagacgaagcgagactggctctggagtggaaagcgagatggggagacagggctgcatgataaatgtcgttagtttctccggtggcaggacgtcagcatatttgctctggctaatggagcaaaagcgacgggcaggtaaagacgtgcattacgttttcatggatacaggttgtgaacatccaatgacatatcggtttgtcagggaagttgtgaagttctgggatataccgctcaccgtattgcaggttgatatcaacccggagcttggacagccaaatggttatacggtatgggaaccaaaggatattcagacgcgaatgcctgttctgaagccatttatcgatatggtaaagaaatatggcactccatacgtcggcggcgcgttctgcactgacagattaaaactcgttcccttcaccaaatactgtgatgaccatttcgggcgagggaattacaccacgtggattggcatcagagctgatgaaccgaagcggctaaagccaaagcctggaatcagatatcttgctgaactgtcagactttgagaaggaagatatcctcgcatggtggaagcaacaaccattcgatttgcaaataccggaacatctcggtaactgcatattctgcattaaaaaatcaacgcaaaaaatcggacttgcctgcaaagatgaggagggattgcagcgtgtttttaatgaggtcatcacgggatcccatgtgcgtgacggacatcgggaaacgccaaaggagattatgtaccgaggaagaatgtcgctggacggtatcgcgaaaatgtattcagaaaatgattatcaagccctgtatcaggacatggtacgagctaaaagattcgataccggctcttgttctgagtcatgcgaaatatttggagggcagcttgatttcgacttcgggagggaagctgcatgatgcgatgttatcggtgcggtgaatgcaaagaagataaccgcttccgaccaaatcaaccttactggaatcgatggtgtctccggtgtgaaagaacaccaacaggggtgttaccactaccgcaggaaaaggaggacgtgtggcgagacagcgacgaagtatcaccgacataatctgcgaaaactgcaaataccttccaacgaaacgcaccagaaataaacccaagccaatcccaaaagaatctgacgtaaaaaccttcaactacacggctcacctgtgggatatccggtggctaagacgtcgtgcgaggaaaacaaggtgattgaccaaaatcgaagttacgaacaagaaagcgtcgagcgagctttaacgtgcgctaactgcggtcagaagctgcatgtgctggaagttcacgtgtgtgagcactgctgcgcagaactgatgagcgatccgaatagctcgatgcacgaggaagaagatgatggctaaaccagcgcgaagacgatgtaaaaacgatgaatgccgggaatggtttcaccctgcattcgctaatcagtggtggtgctctccagagtgtggaaccaagatagcactcgaacgacgaagtaaagaacgcgaaaaagcggaaaaagcagcagagaagaaacgacgacgagaggagcagaaacagaaagataaacttaagattcgaaaactcgccttaaagccccgcagttactggattaaacaagcccaacaagccgtaaacgccttcatcagagaaagagaccgcgacttaccatgtatctcgtgcggaacgctcacgtctgctcagtgggatgccggacattaccggacaactgctgcggcacctcaactccgatttaatgaacgcaatattcacaagcaatgcgtggtgtgcaaccagcacaaaagcggaaatctcgttccgtatcgcgtcgaactgattagccgcatcgggcaggaagcagtagacgaaatcgaatcaaaccataaccgccatcgctggactatcgaagagtgcaaggcgatcaaggcagagtaccaacagaaactcaaagacctgcgaaatagcagaagtgaggccgcatgacgttctcagtaaaaaccattccagacatgctcgttgaagcatacggaaatcagacagaagtagcacgcagactgaaatgtagtcgcggtacggtcagaaaatacgttgatgataaagacgggaaaatgcacgccatcgtcaacgacgttctcatggttcatcgcggatggagtgaaagagatgcgctattacgaaaaaattgatggcagcaaataccgaaatatttgggtagttggcgatctgcacggatgctacacgaacctgatgaacaaactggatacgattggattcgacaacaaaaaagacctgcttatctcggtgggcgatttggttgatcgtggtgcagagaacgttgaatgcctggaattaatcacattcccctggttcagagctgtacgtggaaaccatgagcaaatgatgattgatggcttatcagagcgtggaaacgttaatcactggctgcttaatggcggtggctggttctttaatctcgattacgacaaagaaattctggctaaagctcttgcccataaagcagatgaacttccgttaatcatcgaactggtgagcaaagataaaaaatatgttatctgccacgccgattatccctttgacgaatacgagtttggaaagccagttgatcatcagcaggtaatctggaaccgcgaacgaatcagcaactcacaaaacgggatcgtgaaagaaatcaaaggcgcggacacgttcatctttggtcatacgccagcagtgaaaccactcaagtttgccaaccaaatgtatatcgataccggcgcagtgttctgcggaaacctaacattgattcaggtacagggagaaggcgcatgagactcgaaagcgtagctaaatttcattcgccaaaaagcccgatgatgagcgactcaccacgggccacggcttctgactctctttccggtactgatgtgatggctgctatggggatggcgcaatcacaagccggattcggtatggctgcattctgcggtaagcacgaactcagccagaacgacaaacaaaaggctatcaactatctgatgcaatttgcacacaaggtatcggggaaataccgtggtgtggcaaagcttgaaggaaatactaaggcaaaggtactgcaagtgctcgcaacattcgcttatgcggattattgccgtagtgccgcgacgccgggggcaagatgcagagattgccatggtacaggccgtgcggttgatattgccaaaacagagctgtgggggagagttgtcgagaaagagtgcggaagatgcaaaggcgtcggctattcaaggatgccagcaagcgcagcatatcgcgctgtgacgatgctaatcccaaaccttacccaacccacctggtcacgcactgttaagccgctgtatgacgctctggtggtgcaatgccacaaagaagagtcaatcgcagacaacattttgaatgcggtcacacgttagcagcatgattgccacggatggcaacatattaacggcatgatattgacttattgaataaaattgggtaaatttgactcaacgatgggttaattcgctcgttgtggtagtgagatgaaaagaggcggcgcttactaccgattccgcctagttggtcacttcgacgtatcgtctggaactccaaccatcgcaggcagagaggtctgcaaaatgcaatcccgaaacagttcgcaggtaatagttagagcctgcataacggtttcgggattttttatatctgcacaacaggtaagagcattgagtcgataatcgtgaagagtcggcgagcctggttagccagtgctctttccgttgtgctgaattaagcgaataccggaagcagaaccggatcaccaaatgcgtacaggcgtcatcgccgcccagcaacagcacaacccaaactgagccgtagccactgtctgtcctgaattcattagtaatagttacgctgcggccttttacacatgaccttcgtgaaagcgggtggcaggaggtcgcgctaacaacctcctgccgttttgcccgtgcatatcggtcacgaacaaatctgattactaaacacagtagcctggatttgttctatcagtaatcgaccttattcctaattaaatagagcaaatccccttattgggggtaagacatgaagatgccagaaaaacatgacctgttggccgccattctcgcggcaaaggaacaaggcatcggggcaatccttgcgtttgcaatggcgtaccttcgcggcagatataatggcggtgcgtttacaaaaacagtaatcgacgcaacgatgtgcgccattatcgcctggttcattcgtgaccttctcgacttcgccggactaagtagcaatctcgcttatataacgagcgtgtttatcggctacatcggtactgactcgattggttcgcttatcaaacgcttcgctgctaaaaaagccggagtagaagatggtagaaatcaataatcaacgtaaggcgttcctcgatatgctggcgtggtcggagggaactgataacggacgtcagaaaaccagaaatcatggttatgacgtcattgtaggcggagagctatttactgattactccgatcaccctcgcaaacttgtcacgctaaacccaaaactcaaatcaacaggcgcttaagactggccgtcgttttacaacacagaaagagtttgtagaaacgcaaaaaggccatccgtcaggggccttctgcttagtttgatgcctggcagttccctactctcgccttccgcttcctcgctcactgactcgctgcgctcggtcgttcggctgcggcgagcggtatcagctcactcaaaggcggtaatacggttatccacagaatcaggggataacgcaggaaagaacatgtgagcaaaaggccagcaaaaggccaggaaccgtaaaaaggccgcgttgctggcgtttttccataggctccgcccccctgacgagcatcacaaaaatcgacgctcaagtcagaggtggcgaaacccgacaggactataaagataccaggcgtttccccctggaagctccctcgtgcgctctcctgttccgaccctgccgcttaccggatacctgtccgcctttctcccttcgggaagcgtggcgctttctcatagctcacgctgtaggtatctcagttcggtgtaggtcgttcgctccaagctgggctgtgtgcacgaaccccccgttcagcccgaccgctgcgccttatccggtaactatcgtcttgagtccaacccggtaagacacgacttatcgccactggcagcagccactggtaacaggattagcagagcgaggtatgtaggcggtgctacagagttcttgaagtggtgggctaactacggctacactagaagaacagtatttggtatctgcgctctgctgaagccagttaccttcggaaaaagagttggtagctcttgatccggcaaacaaaccaccgctggtagcggtggtttttttgtttgcaagcagcagattacgcgcagaaaaaaaggatctcaagaagatcctttgatcttttctacggggtctgacgctcagtggaacgacgcgcgcgtaactcacgttaagggattttggtcatgagcttgcgccgtcccgtcaagtcagcgtaatgctctgcttttagaaaaactcatcgagcatcaaatgaaactgcaatttattcatatcaggattatcaataccatatttttgaaaaagccgtttctgtaatgaaggagaaaactcaccgaggcagttccataggatggcaagatcctggtatcggtctgcgattccgactcgtccaacatcaatacaacctattaatttcccctcgtcaaaaataaggttatcaagtgagaaatcaccatgagtgacgactgaatccggtgagaatggcaaaagtttatgcatttctttccagacttgttcaacaggccagccattacgctcgtcatcaaaatcactcgcatcaaccaaaccgttattcattcgtgattgcgcctgagcgaggcgaaatacgcgatcgctgttaaaaggacaattacaaacaggaatcgagtgcaaccggcgcaggaacactgccagcgcatcaacaatattttcacctgaatcaggatattcttctaatacctggaacgctgtttttccggggatcgcagtggtgagtaaccatgcatcatcaggagtacggataaaatgcttgatggtcggaagtggcataaattccgtcagccagtttagtctgaccatctcatctgtaacatcattggcaacgctacctttgccatgtttcagaaacaactctggcgcatcgggcttcccatacaagcgatagattgtcgcacctgattgcccgacattatcgcgagcccatttatacccatataaatcagcatccatgttggaatttaatcgcggcctcgacgtttcccgttgaatatggctcatattcttcctttttcaatattattgaagcatttatcagggttattgtctcatgagcggatacatatttgaatgtatttagaaaaataaacaaataggggtcagtgttacaaccaattaaccaattctgaacattatcgcgagcccatttatacctgaatatggctcataacaccccttgtttgcctggcggcagtagcgcggtggtcccacctgaccccatgccgaactcagaagtgaaacgccgtagcgccgatggtagtgtggggactccccatgcgagagtagggaactgccaggcatcaaataaaacgaaaggctcagtcgaaagactgggcctttcgcccgggctaattagggggtgtcgcccttattcgactctatagtgaagttcctattctctagaaagtataggaacttctgaagtggggtcgacttaattaagg

SEQ ID NO: 10 - DNA, 583 bp, synthetic construct
  misc_feature 1..583: note = constructed sequence
  source 1..583: mol_type = other DNA
cgttacataacttacggtaaatggcccgcctggctgaccgcccaacgacccccgcccattgacgtcaataatgacgtatgttcccatagtaacgccaatagggactttccattgacgtcaatgggtggagtatttacggtaaactgcccacttggcagtacatcaagtgtatcatatgccaagtacgccccctattgacgtcaatgacggtaaatggcccgcctggcattatgcccagtacatgaccttatgggactttcctacttggcagtacatctacgtattagtcatcgctattaacatggtcgaggtgagccccacgttctgcttcactctccccatctcccccccctccccacccccaattttgtatttatttattttttaattattttgtgcagcgatgggggcggggggggggggggggcgcgcgccaggcggggcggggcggggcgaggggcggggcggggcgaggcggagaggtgcggcggcagccaatcagagcggcgcgctccgaaagtttccttttatggcgaggcggcggcggcggcggccctataaaaagcgaagcgcgcggcgggcg

SEQ ID NO: 11 - DNA, 2238 bp, synthetic construct
  misc_feature 1..2238: note = constructed sequence
  source 1..2238: mol_type = other DNA
atggctgccgatggttatcttccagattggctcgaggacactctctctgaaggaataagacagtggtggaagctcaaacctggcccaccaccaccaaagcccgcagagcggcataaggacgacagcaggggtcttgtgcttcctgggtacaagtacctcggacccttcaacggactcgacaagggagagccggtcaacgaggcagacgccgcggccctcgagcacgacaaagcctatgaccggcagctcgacagcggagacaacccgtacctcaagtacaaccacgccgacgcggagtttcaggagcgccttaaagaagatacgtcttttgggggcaacctcggacgagcagtcttccaggcgaaaaagagggttcttgaacctctgggcctggttgaggaacctgttaagacggctccgggaaaaaagaggccggtagagcactctcctgtggagccagactcctcctcgggaaccggaaaggcgggccagcagcctgcaagaaaaagattgaattttggtcagactggagacgcagactcagtacctgacccccagcctctcggacagccaccagcagccccctctggtctgggaactaatacgatggctacaggcagtggcgcaccaatggcagacaataacgagggcgccgacggagtgggtaattcctcgggaaattggcattgcgattccacatggatgggcgacagagtcaccaccaccagcacccgaacctgggccctgcccacctacaacaaccacctctacaaacaaatttccagccaatcaggagcctcgaacgacaatcactactttggctacagcaccccttgggggtattttgacttcaacagattccactgccacttttcaccacgtgactggcaaagactcatcaacaacaactggggattccgacccaagagactcaacttcaagctctttaacattcaagtcaaagaggtcacgcagaatgacggtacgacgacgattgccaataaccttaccagcacggttcaggtgtttactgactcggagtaccagctcccgtacgtcctcggctcggcgcatcaaggatgcctcccgccgttcccagcagacgtcttcatggtgccacagtatggatacctcaccctgaacaacgggagtcaggcagtaggacgctcttcattttactgcctggagtactttccttctcagatgctgcgtaccggaaacaactttaccttcagctacacttttgaggacgttcctttccacagcagctacgctcacagccagagtctggaccgtctcatgaatcctctcatcgaccagtacctgtattacttgagcagaacaaacactccaagtggaaccaccacgcagtcaaggcttcagttttctcaggccggagcgagtgacattcgggaccagtctaggaactggcttcctggaccctgttaccgccagcagcgagtatcaaagacatctgcggataacaacaacagtgaatactcgtggactggagctaccaagtaccacctcaatggcagagactctctggtgaatccgggcccggccatggcaagccacaaggacgatgaagaaaagttttttcctcagagcggggttctcatctttgggaagcaaggctcagagaaaacaaatgtggacattgaaaaggtcatgattacagacgaagaggaaatcaggacaaccaatcccgtggctacggagcagtatggttctgtatctaccaacctccagagaggcaacctagcactcggcgaaacaacaagacctgctaggcaagcagctaccgcagatgtcaacacacaaggcgttcttccaggcatggtctggcaggacagagatgtgtaccttcaggggcccatctgggcaaagattccacacacggacggacattttcacccctctcccctcatgggtggattcggacttaaacaccctcctccccagattctcatcaagaacaccccggtacctgcgaatccttcgaccaccttcagtgcggcaaagtttgcttccttcatcacacagtactccacgggacaggtcagcgtggagatcgagtgggagctgcagaaggaaaacagcaaacgctggaatcccgaaattcagtacacttccaactacaacaagtctattaatgtggactttactgtggacactaatggcgtgtattcagagcctcgccccattggcaccagatacctgactcgtaatctgtaa

SEQ ID NO: 12 - protein, 740 aa, synthetic construct
  REGION 1..740: note = constructed sequence
MAADGYLPDWLEDTLSEGIRQWWKLKPGPPPPKPAERHKDDSRGLVLPGYKYLGPFNGLDKGEPVNEADAAALEHDKAYDRQLDSGDNPYLKYNHADAEFQERLKEDTSFGGNLGRAVFQAKKRVLEPLGLVEEPVKTAPGKKRPVEHSPVEPDSSSGTGKAGQQPARKRLNFGQTGDADSVPDPQPLGQPPAAPSGLGTNTMATGSGAPMADNNEGADGVGNSSGNWHCDSTWMGDRVTTTSTRTWALPTYNNHLYKQISSQSGASNDNHYFGYSTPWGYFDFNRFHCHFSPRDWQRLINNNWGFRPKRLNFKLFNIQVKEVTQNDGTTTIANNLTSTVQVFTDSEYQLPYVLGSAHQGCLPPFPADVFMVPQYGYLTLNNGSQAVGRSSFYCLEYFPSQMLRTGNNFTFSYTFEDVPFHSSYAHSQSLDRLMNPLIDQYLYYLSRTNTPSGTTTQSRLQFSQAGASDIRDQSRNWLPGPCYRQQRVSKTSADNNNSEYSWTGATKYHLNGRDSLVNPGPAMASHKDDEEKFFPQSGVLIFGKQGSEKTNVDIEKVMITDEEEIRTTNPVATEQYGSVSTNLQRGNLALGETTRPARQAATADVNTQGVLPGMVWQDRDVYLQGPIWAKIPHTDGHFHPSPLMGGFGLKHPPPQILIKNTPVPANPSTTFSAAKFASFITQYSTGQVSVEIEWELQKENSKRWNPEIQYTSNYNKSINVDFTVDTNGVYSEPRPIGTRY

SEQ ID NO: 13 - DNA, 20 bp, synthetic construct
  misc_feature 1..20: note = constructed sequence
  source 1..20: mol_type = other DNA
gcctgttcctgcttgcttac

SEQ ID NO: 14 - DNA, 22 bp, synthetic construct
  misc_feature 1..22: note = constructed sequence
  source 1..22: mol_type = other DNA
tgctttccaaagtaagcacaaa

SEQ ID NO: 15 - DNA, 20 bp, synthetic construct
  misc_feature 1..20: note = constructed sequence
  source 1..20: mol_type = other DNA
cctggcctccagacaagtag